European Patent Application EP 4 461 819 A1, published November 13, 2024. Title: Method for eliminating carryover contamination in nucleic acid amplification reaction using uracil-DNA glycosylase derived from Photobacterium leiognathi. Applicant: 주식회사 씨젠. The sequence listing filed with the application follows.

SEQUENCE LISTING (12 sequences)

SEQ ID NO: 1 - DNA, 663 bp, Photobacterium leiognathi
  source 1..663: mol_type = genomic DNA
atgaccgccagttggtctacttttatagcgcagcaacaagcgcaagcgtatttcatcgatattgagcaggcagtcgatgctgctcgtcatgctggtaaagtggtttatcctcctcaagaagatgtctttaatgcgtttaccagtacgccacttgagaaaaccaaagtcgtgatattaggtcaagatccgtatcacggacctaagcaagcccatggtcttagcttctcggtattgccaggtgtgaaaacaccgccgtcactggcaaatatgtataaagagttagccactgatatcgacggttttactactccagaacatggttatttacagccatgggctgagcaaggtgtgttgttattaaatacggtattaactgtcgagcagggtaatgctcactcacacgctaagattggttgggaaacttttactaatcgcgcgattgaatatatcaatgataatactgaaggcgtgattttcttgttgtggggcgcacatgcgcaaaagaaaggtaagaagatagatacaacgcgtcaccacgtattgcattcagcgcacccgtcaccgttatcggcttatcgtggtttctttggttgccaacatttctctaaaacaaatcagttattagctgagatggggaaagcaccgatcaattggcaaatataa

SEQ ID NO: 2 - protein, 220 aa, Photobacterium leiognathi
MTASWSTFIAQQQAQAYFIDIEQAVDAARHAGKVVYPPQEDVFNAFTSTPLEKTKVVILGQDPYHGPKQAHGLSFSVLPGVKTPPSLANMYKELATDIDGFTTPEHGYLQPWAEQGVLLLNTVLTVEQGNAHSHAKIGWETFTNRAIEYINDNTEGVIFLLWGAHAQKKGKKIDTTRHHVLHSAHPSPLSAYRGFFGCQHFSKTNQLLAEMGKAPINWQI

SEQ ID NO: 3 - DNA, 20 bp, synthetic construct
  source 1..20: mol_type = other DNA
ggnccrgayccntaycaygg

SEQ ID NO: 4 - DNA, 23 bp, synthetic construct
  source 1..23: mol_type = other DNA
ttyttytgngcrtgngmncccca

SEQ ID NO: 5 - DNA, 21 bp, synthetic construct
  source 1..21: mol_type = other DNA
aagaccatgggcttgcttagg

SEQ ID NO: 6 - DNA, 23 bp, synthetic construct
  source 1..23: mol_type = other DNA
tcaatgataatactgaaggcgtg

SEQ ID NO: 7 - DNA, 28 bp, synthetic construct
  source 1..28: mol_type = other DNA
nnnnncatatgaccgccagttggtctac

SEQ ID NO: 8 - DNA, 36 bp, synthetic construct
  source 1..36: mol_type = other DNA
nnnnnctcgagtatttgccaattgatcggtgctttc

SEQ ID NO: 9 - DNA, 20 bp, synthetic construct
  source 1..20: mol_type = other DNA
aataacgtcggcaactttgg

SEQ ID NO: 10 - DNA, 20 bp, synthetic construct
  source 1..20: mol_type = other DNA
gttacgccaccagtcatcct

SEQ ID NO: 11 - DNA, 20 bp, synthetic construct
  source 1..20: mol_type = other DNA
caaaggcggttaaggtggta

SEQ ID NO: 12 - DNA, 20 bp, synthetic construct
  source 1..20: mol_type = other DNA
ggctgtaccggacaatgagt